European Patent Specification EP 3 608 413 B1, published March 15, 2023. Title: USE OF NON-AGROBACTERIUM BACTERIAL SPECIES FOR PLANT TRANSFORMATION. Applicant: Monsanto Technology, LLC. The sequence listing filed with the application follows.

SEQUENCE LISTING (30 sequences)

SEQ ID NO: 1 - DNA, 21 bp, Artificial Sequence
  Description of Artificial Sequence:  Synthetic Primer
gagagtttgatcctggctcag

SEQ ID NO: 2 - DNA, 21 bp, Artificial Sequence
  Description of Artificial Sequence:  Synthetic Primer
aaggaggtgatccagccgcag

SEQ ID NO: 3 - DNA, 30 bp, Artificial Sequence
  Description of Artificial Sequence:  Synthetic Primer
acaataatgtgtgttgttaagtcttgttgc

SEQ ID NO: 4 - DNA, 28 bp, Artificial Sequence
  Description of Artificial Sequence:  Synthetic Primer
ctcaaacctacactcaatatttggtgag

SEQ ID NO: 5 - DNA, 24 bp, Artificial Sequence
  Description of Artificial Sequence:  Synthetic Primer
agatctggctcgcggcggacgcac

SEQ ID NO: 6 - DNA, 24 bp, Artificial Sequence
  Description of Artificial Sequence:  Synthetic Primer
cgctcgcgtcattctttgctggag

SEQ ID NO: 7 - DNA, 23 bp, Artificial Sequence
  Description of Artificial Sequence:  Synthetic Primer
tcagcaggatgacgccgttatcg

SEQ ID NO: 8 - DNA, 23 bp, Artificial Sequence
  Description of Artificial Sequence:  Synthetic Primer
tctcgcccgaccaataccaacac

SEQ ID NO: 9 - DNA, 31 bp, Artificial Sequence
  Description of Artificial Sequence:  Synthetic Primer
gctgacgggcccggatgaatgtcagctactg

SEQ ID NO: 10 - DNA, 42 bp, Artificial Sequence
  Description of Artificial Sequence:  Synthetic Primer
gctctagaaattgtaagcgttaataattcagaagaactcgtc

SEQ ID NO: 11 - DNA, 28 bp, Artificial Sequence
  Description of Artificial Sequence:  Synthetic Primer
caattgcatttggctcttaattatctgg

SEQ ID NO: 12 - DNA, 26 bp, Artificial Sequence
  Description of Artificial Sequence:  Synthetic Primer
gcatgcccgatcgcgctcaagtaatc

SEQ ID NO: 13 - DNA, 23 bp, Artificial Sequence
  Description of Artificial Sequence:  Synthetic Primer
tctaggtccccccgcgcccatcg

SEQ ID NO: 14 - DNA, 28 bp, Artificial Sequence
  Description of Artificial Sequence:  Synthetic Primer
ccatggatctttctggcaatgagaaatc

SEQ ID NO: 15 - DNA, 28 bp, Artificial Sequence
  Description of Artificial Sequence:  Synthetic Primer
gtcaaaagctgttgacgctttggctacg

SEQ ID NO: 16 - DNA, 23 bp, Artificial Sequence
  Description of Artificial Sequence:  Synthetic Primer
acgggagaggcggtgttagttgc

SEQ ID NO: 17 - DNA, 23 bp, Artificial Sequence
  Description of Artificial Sequence:  Synthetic Primer
cgatagcgacaatgccgagaacg

SEQ ID NO: 18 - DNA, 24 bp, Artificial Sequence
  Description of Artificial Sequence:  Synthetic Primer
atgcccgatcgagctcaagttatc

SEQ ID NO: 19 - DNA, 24 bp, Artificial Sequence
  Description of Artificial Sequence:  Synthetic Primer
tgaaaggacacctctccgttgctg

SEQ ID NO: 20 - DNA, 27 bp, Artificial Sequence
  Description of Artificial Sequence:  Synthetic Primer
ccatggatccgaaggccgaaggcaatg

SEQ ID NO: 21 - DNA, 23 bp, Artificial Sequence
  Description of Artificial Sequence:  Synthetic Primer
ctacagactgtttacggttgggc

SEQ ID NO: 22 - DNA, 23 bp, Artificial Sequence
  Description of Artificial Sequence:  Synthetic Primer
gtgagcaaagccgctgccatatc

SEQ ID NO: 23 - DNA, 23 bp, Artificial Sequence
  Description of Artificial Sequence:  Synthetic Primer
tagagcgtctgcttggttaaacc

SEQ ID NO: 24 - DNA, 1490 bp, A. tumefaciens
tagaaaggaggtgatccagccgcaggttcccctacggctaccttgttacgacttcaccccagtcgctgaccctaccgtggttagctgcctccttgcggttagcgcactaccttcgggtaaaaccaactcccatggtgtgacgggcggtgtgtacaaggcccgggaacgtattcaccgcagcatgctgatctgcgattactagcgattccaacttcatgcactcgagttgcagagtgcaatccgaactgagatggcttttggagattagctcgacatcgctgtctcgctgcccactgtcaccaccattgtagcacgtgtgtagcccagcccgtaagggccatgaggacttgacgtcatccccaccttcctctcggcttatcaccggcagtccccttagagtgcccaactaaatgctggcaactaagggcgagggttgcgctcgttgcgggacttaacccaacatctcacgacacgagctgacgacagccatgcagcacctgttctggggccagcctaactgaaggacatcgtctccaatgcccataccccgaatgtcaagagctggtaaggttctgcgcgttgcttcgaattaaaccacatgctccaccgcttgtgcgggcccccgtcaattcctttgagttttaatcttgcgaccgtactccccaggcggaatgtttaatgcgttagctgcgccaccgaacagtatactgcccgacggctaacattcatcgtttacggcgtggactaccagggtatctaatcctgtttgctccccacgctttcgcacctcagcgtcagtaatggaccagtaagccgccttcgccactggtgttcctccgaatatctacgaatttcacctctacactcggaattccacttacctcttccatactcaagatacccagtatcaaaggcagttccgcagttgagctgcgggatttcacccctgacttaaatatccgcctacgtgcgctttacgcccagtaattccgaacaacgctagcccccttcgtattaccgcggctgctggcacgaagttagccggggcttcttctccgactaccgtcattatcttcatcggtgaaagagctttacaaccctaaggccttcatcactcacgcggcatggctggatcaggcttgcgcccattgtccaatattccccactgctgcctcccgtaggagtttgggccgtgtctcagtcccaatgtggctgatcatcctctcagaccagctatggatcgtcgccttggtaggcctttaccccaccaactagctaatccaacgcgggctcatccatccccgataaatctttcccccgtagggcgtatgcggtattaattccagtttcccagagctattccgcagagatgggtagattcccacgcgttactcacccgtctgccactccccttgcggggcgttcgacttgcatgtgttaagcctgccgccagcgttcgttctgagccaggatcaaactctcaagttgag

SEQ ID NO: 25 - DNA, 1366 bp, Rhizobium leguminosarum
cttcgcccagtcgctgaccckascgkggttagctgsctcckkgcggttagcgcactaccttcgggtaaaaccaactcccatggtgtgacgggcggtgtgtacaaggcccgggaacgtattcaccgcggcatgctgatccgcgattactagcgattccaacttcatgcactcgagttgcagagtgcaatccgaactgaratggcttttggagattagctcacactcgcgtgctcgctgcccactgtcaccaccattgtagcacgtgtgtagcccagcccgtaagggccatgaggacttgacgtcatcmccaccttcctctcggcttatcaccggcagtccccttagagtgcccaactgaatgctggcaactaagggcgagggttgcgctcgttgcgggacttaacccaacatctcacgacacgagctgacgacagccatgcagcacctgtgtcccggtccccgaagggaaccttgcatctctgcaagtagccgggcatgtcaagggctggtaaggttctgcgcgttgcttcgaattaaaccacatgctccaccgcttgtgcgggcccccgtcaattcctttgagttttaatcttgcgaccgtactccccaggcggaatgtttaatgcgttagctgcgccaccgaacagtatactgcccgacggctaacattcatcgtttacggcgtggactaccagggtatctaatcctgtttgctccccacgctttcgcacctcagcgtcagtaatggaccagtgagccgccttcgccactggtgttcctccgaatatctacgaatttcacctctacactcggaattccactcacctcttccatactccagatcgacagtatcaaaggcagttccagggttgagccctgggatttcacccctgactgatcgatccgcctacgtgcgctttacgcccagtaattccgaacaacgctagcccccttcgtattaccgcggctgctggcacgaagttagccggggcttcttctccggataccgtcattatcttctccggtgaaagagctttacaaccctagggccttcatcactcacgcggcatggctggatcaggcttgcgcccattgtccaatattccccactgctgcctcccgtaggagtttgggccgtgtctcagtcccaatgtggctgatcatcctctcagaccagctatggatcgtcgccttggtaggcctttaccccaccaactagctaatccaacgcgggctcatccttgaccgataaatctttctcccgaaggacacatacggtattagcacaagtttccctgcgttattccgtagtcaagggtagattcccacgcgttactcacccgtctgccgctccccttgcggggcg

SEQ ID NO: 26 - DNA, 1323 bp, Rhizobium leguminosarum
agcgcactacctctcgggtaaaaccaactcccatggtgtgacgggcggtgtgtacaaggcccgggaacgtattcaccgcggcatgctgatccgcgattactagcgattccaacttcatgcactcgagttgcagagtgcaatccgaactgagatggcttttggagattagctcacactcgcgtgctcgctgcccactgtcaccaccattgtagcacgtgtgtagcccagcccgtaagggccatgaggacttgacgtcawcaccaccttcctctcggcttatcaccggcagtccccttagagtgcccaactgaatgctggcaactaagggcgagggttgcgctcgttgcgggacttaacccaacatctcacgacacgagctgacgacagccatgcagcacctgtgtcccggtccccgaagggaccttgcatctctgcaagtagcgggcatgtcaagggctggtaaggttctgcgcgttgcttcgaattaaaccacatgctccaccgcttgtgcgggcccccgtcaattccttgagttttaatcttgcgaccgtactccccaggcggaatgtttaatgcgttagctgcgccaccgaacagtatactgcccgacggctaacattcatcgtttacggcgtggactaccagggtatctaatcctgtttgctccccacgctttcgcacctcagcgtcagtaatggaccagtgagccgccttcgccactggtgttcctccgaatatctacgaatttcacctctacactcggaattccactcacctcttccatactccagatcgacagtatcaaaggcagttccagggttgagccctgggatttcacccctgactgatcgatccgcctacgtgcgctttacgcccagtaattccgaacaacgctagcccccttcgtattaccgcggctgctggcacgaagttagccggggcttcttctccggataccgtcattatcttctccggtgaaagagctttacaaccctagggccttcatcactcacgcggcatggctkgatcaggcttgcgcccattgtccaatattccccactgctgcctcccgtaggagtttgggccgtgtctcagtcccaatgtggctgatcatcctctcagaccagctatggatcgtcgccttggtaggcctttaccccaccaactagctaatccaacgcgggctcatccttgaccgataaatctttctcccgaaggacacatacggtattagcacaagtttccctgcgttattccgtagtcaagggtagattcccacgcgttactcacccgtctgccgcttccccttgcggggcgcatacg

SEQ ID NO: 27 - DNA, 1341 bp, Rhizobium leguminosarum
ggttagctgcctccttgcggttagcgcactaccttcgggtaaaaccaactcccatggtgtgacgggcggtgtgtacaaggcccgggaacgtattcaccgcggcatgctgatccgcgattacgaccgattccaacttctagcactcgagttgcagagtgcaatccgaactgagatggcttttggagattagctcacactcgcgtgctcgctgcccactgtcaccaccattgtagcacgtgtgtagcccagcccgtaagggccatgaggacttgacgtcatccccaccttcctctcggcttatcaccggcagtccccttagagtgcccaactgaatgctggcaactaagggcgagggttgcgctcgttgcgggacttaacccaacatctcacgacacgagctgacgacagccatgcagcacctgtgtcccggtccccgaagggaaccttgcatctctgcaagtagccgggcatgtcaagggctggtaaggttctgcgcgttgcttcraattaaaccacatgctccaccgcttgtgcgggcccccgtcaattcctttgagttttaatcttgcgaccgtactccccaggcggaatgtttaatgcgttagctgcgccaccgaacagtatactgcccgacggctaacattcatcgtttacggcgtggactaccagggtatctaatcctgtttgctccccacgctttcgcacctcagcgtcagtaatggaccagtgagccgccttcgccactggtgttcctccgaatatctacgaatttcacctctacactcggaattccactcacctcttccatactccagatcgacagtatcaaaggcagttccagggttgagccctgggatttcacccctgactgatcgatccgcctacgtgcgctttacgcccagtaattccgaacaacgctagcccccttcgtattaccgcggctgctggcacgaagttagccggggcttcttctccggataccgtcattatcttctccggtgaaagagctttacaaccctagggccttcatcactcacgcggcatggctggatcaggcttgcgcccattgtccaatattccccactgctgcctcccgtaggagtttgggccgtgtctcagtcccaatgtggctgatcatcctctcagaccagctatggatcgtcgccttggtaggcctttaccccaccaactagctaatccaacgcgggccgatcctttaccgataaatctttcccccgaagggcacatacggtattagcacaagtttccctgcgttattccgtagtaaagggtacgttcccacgcgttactcacccgtctgccgctccccttgcgtggcgc

SEQ ID NO: 28 - DNA, 1341 bp, Mesorhizobium loti
ccttgcggttagcacagcgccttcgggtaaaaccaactcccatggtgtgacgggcggtgtgtacaaggcccgggaacgtattcaccgcggcatgctgatccgcgattactagcgattccaacttcatgcactcgagttgcagagtgcaatccgaactgagatggcttttggagattagctcgacctcgcggtctcgctgcccactgtcaccaccattgtagcacgtgtgtagcccagcccgtaagggccatgaggacttgacgtcatccccaccttcctctcggcttatcaccggcagtccccttagagtgcccaactgaatgctggcaactaagggcgagggttgcgctcgttgcgggacttaacccaacatctcacgacacgagctgacgacagccatgcagcacctgtcaccggtccagccgaactgaaggtatccatctctggaaaccgcgaccgggatgtcaagggctggtaaggttctgcgcgttgcttcgaattaaaccacatgctccaccgcttgtgcgggcccccgtcaattcctttgagttttaatcttgcgaccgtactccccaggcgggaagcttaatgcgttagctgcgccaccgacaagtaaacttgccaacggctagcttccatcgtttacggcgtggactaccagggtatctaatcctgtttgctccccacgctttcgcacctcagcgtcagtaccggaccagtgagccgccttcgccactggtgttcctccgaatatctacgaatttcacctctacactcggaattccactcacctcttccggactcgagatacccagtatcaaaggcagttccggggttgagccccgggatttcacccctgacttaagtatccgcctacgtgcgctttacgcccagtaattccgaacaacgctagcccccttcgtattaccgcggctgctggcacgaagttagccggggcttcttctacggttaccgtcattatcttcaccgttgaaagagctttacaaccctagggccttcatcactcacgcggcatggctggatcaggcttgcgcccattgtccaatattccccactgctgcctcccgtaggagtctgggccgtgtctcagtcccagtgtggctgatcatcctctcagaccagctatggatcgtcgccttggtaggccattaccccaccaactagctaatccaacgcgggctcatccatctccgataaatctttctccaaaaggacgtatacggtattagctccagtttcccggagttgttccgtagagatgggtagattcccacgcgttactcacccgtctgccgctccccttgcggggcacgcgccctt

SEQ ID NO: 29 - DNA, 1339 bp, S. Fredii
agccttgcggttagcgcactaccttcgggtagaaccaactcccatggtgtgacgggcggtgtgtamaaggcccgggaacgtattcaccgcagcatgctgatctgcgattactagcgattccaacttcatgcactcgagttgcagagtgcaatccgaactgagatggcttttggagattagctcgacctcgcggtctcgctgcccactgtcaccaccattgtascacgtgtgtagcccagcccgtaagggccatgaggacttgacgtcatccccaccttcctctcggcttatcaccggcagtccccttagagtgaccaactaaatgctggcaactaagggcgagggttgcgctcgttgcgggacttaacccaacatctcacgacacgagctgacgacagccatgcagcacctgtctccgatccagccgaactgaaggatacgatctctcgtatccgcgatcgggatgtcaagggctggtaaggttctgcgcgttgcttcgaattaaaccacatgctccaccgcttgtgcgggcccccgtcaattcctttgagttttaatcttgcgaccgtactccccaggcggaatgtttaatgcgttagctgcgccaccgaacagtaaactgcccgacggctaacattcatcgtttacggcgtggactaccagggtatctaatcctgtttgctccccacgctttcgcacctcagcgtcagtaccggaccagtgagccgccttcgccactggtgttcctccgaatatctacgaatttcacctctacactcggaattccactcacctcttccggactctagacacccagtatcaaaggcagttccggggttgagccccgggatttcacccctgacttaaatgtccgcctacgtgcgctttacgcccagtaattccgaacaacgctagcccccttcgtattaccgcggctgctggcacgaagttagccggggcttcttctccggttaccgtcattatcttcaccggtgaaagagctttacaaccctagggccttcatcactcacgcggcatggctggatcaggcttgcgcccattgtccaatattccccactgctgcctcccgtaggagtttgggccgtgtctcagtcccaatgtggctgatcatcctctcagaccagctatggatcgtcgccttggtaggcctttaccccaccaactagctaatccaacgcgggctcatcctttcccgataaatctttcccccgaagggctcatacggtattagcacaagtttccctgcgttattccgtagaaaagggtagattcccacgcgttactcaccmatctgccgcycccccgcrgcgcgctcccc

SEQ ID NO: 30 - DNA, 1368 bp, Bradyrhizobium sp.
gaaggtaccgtggccggctgcctacctagcgggttagcgcaccgtcttcaggtaaaaccaactcccatggtgtgacgggcggtgtgtacaaggcccgggaacgtattcaccgtggcgtgctgatccacgattactagcgattccaacttcatgggctcgagttgcagagcccaatccgaactgagacggctttttgagatttgcgaagggtcgccccttagcatcccattgtcaccgccattgtagcacgtgtgtagcccagcccgtaagggccatgaggacttgacgtcatccccaccttcctcgcggcttatcaccggcagtctccttagagtgctcaactaaatggtagcaactaaggacgggggttgcgctcgttgcgggacttaacccaacatctcacgacacgagctgacgacagcatgcagcacctgtgctccaggctccgaagagaaggtcacatctctgcgaccggtcctggacatgtcaagggctggtaaggttctgcgcgttgcgtcgaattaaaccacatgctccaccgcttgtgcgggcccccgtcaattccttgagttttaatcttgcgaccgtactccccaggcggaatgcttaaagcgttagctgcgccactagtgagtaaacccactaacggctggcattcatcgtttacggcgtggactaccagggtatctaatcctgtttgctccccacgctttcgtgcctcagcgtcagtatcgggccagtgagccgccttcgccactggtgttcttgcgaatatctacgaatttcacctctacactcgcagttccactcacctctcccgaactcaagatcctcagtatcaaaggcagttctggagttgagctccaggatttcacccctgacttaaagacccgcctacgcaccctttacgcccagtgattccgagcaacgctagcccccttcgtattaccgcggctgctggcacgaagttagccggggcttattcttgcggtaccgtcattatcttcccgcacaaaagagctttacaaccctagggccttcatcactcacgcggcatggctggatcagggttgcccccattgtccaatattccccactgctgcctcccgtaggagtttgggccgtgtctcagtcccaatgtggctgatcatcctctcagaccagctactgatcgtcgccttggtgagccattacctcaccaactagctaatcagacgcgggccgatctttcggcgataaatctttccccgtaagggcttatccggtattagcacaagtttccctgtgttgttccgaaccaaaaggtacgttcccacgcgttactcacccgtctgccgctgacgtatgctwcgcccgckcgccckccct